European Patent Application EP 4 293 103 A1, published December 20, 2023. Title: BIFIDOBACTERIUM ANIMALIS SUBSP. LACTIS AND USE THEREOF. Applicant: WISBIOM (BEIJING) BIOTECHNOLOGY CO., LTD. Application EP22752363.6. The sequence listing filed with the application follows.

SEQUENCE LISTING (4 sequences)

SEQ ID NO: 1 - DNA, 67 bp, Artificial Sequence
  misc_feature (59)..(59): n is a, g, c or t
  misc_feature (60)..(60): b is g, c or t
  misc_feature (64)..(64): s is g or c
tcgtcggcagcgtcagatgtgtataagagacagcctacgggaggcagcagcctacgggnbgcascag

SEQ ID NO: 2 - DNA, 56 bp, Artificial Sequence
  misc_feature (42)..(42): n is a, g, c or t
  misc_feature (43)..(43): v is a, g or c
gtctcgtgggctcggagatgtgtataagagacagtgactacnvgggtatctaatcc

SEQ ID NO: 3 - DNA, 17 bp, Artificial Sequence
  misc_feature (5)..(5): y is c or t
  misc_feature (9)..(9): r is a or g
  misc_feature (10)..(10): b is c, t or g
  misc_feature (14)..(14): s is c or g
cctaygggrbgcascag

SEQ ID NO: 4 - DNA, 20 bp, Artificial Sequence
  misc_feature (8)..(8): n is a, c, g or t
  misc_feature (9)..(9): n is a, c, g or t
ggactacnngggtatctaat